European Patent Application EP 4 180 521 A1, published May 17, 2023. Title: METHOD FOR PRODUCING SURFACE PROTEIN ANTIGEN OF VARICELLA ZOSTER VIRUS. Applicant: GREEN CROSS CORPORATION. The sequence listing filed with the application follows.

SEQUENCE LISTING (4 sequences)

SEQ ID NO: 1 - protein, 537 aa, Artificial Sequence
  MGgE antigen
MGTVNKPVVGVLMGFGIITGTLRITNPVRASVLRYDDFHTDEDKLDTNSVYEPYYHSDHAESSWVNRGESSRKAYDHNSPYIWPRNDYDGFLENAHEHHGVYNQGRGIDSGERLMQPTQMSAQEDLGDDTGIHVIPTLNGDDRHKIVNVDQRQYGDVFKGDLNPKPQGQRLIEVSVEENHPFTLRAPIQRIYGVRYTETWSFLPSLTCTGDAAPAIQHICLKHTTCFQDVVVDVDCAENTKEDQLAEISYRFQGKKEADQPWIVVNTSTLFDELELDPPEIEPGVLKVLRTEKQYLGVYIWNMRGSDGTSTYATFLVTWKGDEKTRNPTPAVTPQPRGAEFHMWNYHSHVFSVGDTFSLAMHLQYKIHEAPFDLLLEWLYVPIDPTCQPMRLYSTCLYHPNAPQCLSHMNSGCTFTSPHLAQRVASTVYQNCEHADNYTAYCLGISHMEPSFGLILHDGGTTLKFVDTPESLSGLYVFVVYFNGHVEAVAYTVVSTVDHFVNAIEERGFPPTAGQPPATTKPKEITPVNPGTSPLLR

SEQ ID NO: 2 - DNA, 1610 bp, Artificial Sequence
  MGgE antigen
atgggaacagtcaacaaaccagtcgtcggcgtgctgatgggcttcggtattattacaggaactctgaggattactaaccccgtgcgcgcctctgtgctgcggtacgacgatttccacacagacgaggataagctggacaccaattccgtgtatgagccctactatcactctgatcacgccgagagctcctgggtgaaccggggcgagtctagcaggaaggcttacgaccacaacagcccttatatctggccacggaatgactacgatggctttctggagaacgcccacgagcaccacggcgtgtataatcagggcagaggcatcgactctggcgagcggctgatgcagcccacccagatgagcgcccaggaggatctgggcgacgatacaggcatccacgtgatccctaccctgaatggcgacgataggcacaagatcgtgaacgtggatcagagacagtacggcgacgtgttcaagggcgatctgaatcccaagcctcagggccagaggctgatcgaggtgtccgtggaggagaaccaccccttcaccctgagagcccctatccagcggatctacggcgtgaggtataccgagacatggagctttctgccatccctgacatgcaccggcgacgctgctcctgctatccagcacatctgcctgaagcacaccacatgttttcaggacgtggtggtggacgtggattgtgccgagaatacaaaggaggatcagctggctgagatctcctaccggttccagggcaagaaggaggccgatcagccttggatcgtggtgaacacctctacactgtttgacgagctggagctggatccccctgagatcgagccaggcgtgctgaaggtgctgagaaccgagaagcagtacctgggcgtgtatatctggaacatgcggggctctgacggcaccagcacatacgctaccttcctggtcacatggaagggcgatgagaagacccggaatccaacacctgctgtgacccctcagccaaggggagctgagtttcacatgtggaactatcactcccacgtgttctctgtgggcgacacctttagcctggccatgcacctgcaatataagatccacgaggctcctttcgacctgctgctggagtggctgtatgtgcccatcgatcctacatgccagccaatgaggctgtactccacctgtctgtatcacccaaatgccccccaatgcctgagccacatgaactccggctgtacctttacaagcccccacctggcccagagagtggcttccacagtgtaccagaactgcgagcacgccgacaattacaccgcttattgtctgggcatctctcacatggagcccagcttcggcctgatcctgcacgacggcggcaccacactgaagtttgtggatacacccgagtccctgtctggcctctacgtgttcgtggtgtacttcaacggccacgtggaggccgtggcttatacagtggtgtctaccgtggatcacttcgtgaacgccatcgaggagagaggatttccacctaccgctggacagcctccagctaccacaaagcctaaggaaatcacccctgtcaatcctggaacttcacctctgctgcg

SEQ ID NO: 3 - protein, 623 aa, Artificial Sequence
  VZV gE antigen
MGTVNKPVVGVLMGFGIITGTLRITNPVRASVLRYDDFHTDEDKLDTNSVYEPYYHSDHAESSWVNRGESSRKAYDHNSPYIWPRNDYDGFLENAHEHHGVYNQGRGIDSGERLMQPTQMSAQEDLGDDTGIHVIPTLNGDDRHKIVNVDQRQYGDVFKGDLNPKPQGQRLIEVSVEENHPFTLRAPIQRIYGVRYTETWSFLPSLTCTGDAAPAIQHICLKHTTCFQDVVVDVDCAENTKEDQLAEISYRFQGKKEADQPWIVVNTSTLFDELELDPPEIEPGVLKVLRTEKQYLGVYIWNMRGSDGTSTYATFLVTWKGDEKTRNPTPAVTPQPRGAEFHMWNYHSHVFSVGDTFSLAMHLQYKIHEAPFDLLLEWLYVPIDPTCQPMRLYSTCLYHPNAPQCLSHMNSGCTFTSPHLAQRVASTVYQNCEHADNYTAYCLGISHMEPSFGLILHDGGTTLKFVDTPESLSGLYVFVVYFNGHVEAVAYTVVSTVDHFVNAIEERGFPPTAGQPPATTKPKEITPVNPGTSPLIRYAAWTGGLAAVVLLCLVIFLICTAKRMRVKAYRVDKSPYNQSMYYAGLPVDDFEDSESTDTEEEFGNAIGGSHGGSSYTVYIDKTR

SEQ ID NO: 4 - protein, 546 aa, Artificial Sequence
  GSKgE
MGTVNKPVVGVLMGFGIITGTLRITNPVRASVLRYDDFHIDEDKLDTNSVYEPYYHSDHAESSWVNRGESSRKAYDHNSPYIWPRNDYDGFLENAHEHHGVYNQGRGIDSGERLMQPTQMSAQEDLGDDTGIHVIPTLNGDDRHKIVNVDQRQYGDVFKGDLNPKPQGQRLIEVSVEENHPFTLRAPIQRIYGVRYTETWSFLPSLTCTGDAAPAIQHICLKHTTCFQDVVVDVDCAENTKEDQLAEISYRFQGKKEADQPWIVVNTSTLFDELELDPPEIEPGVLKVLRTEKQYLGVYIWNMRGSDGTSTYATFLVTWKGDEKTRNPTPAVTPQPRGAEFHMWNYHSHVFSVGDTFSLAMHLQYKIHEAPFDLLLEWLYVPIDPTCQPMRLYSTCLYHPNAPQCLSHMNSGCTFTSPHLAQRVASTVYQNCEHADNYTAYCLGISHMEPSFGLILHDGGTTLKFVDTPESLSGLYVFVVYFNGHVEAVAYTVVSTVDHFVNAIEERGFPPTAGQPPATTKPKEITPVNPGTSPLIRYAAWTGGLA